European Patent Application EP 4 541 908 A1, published April 23, 2025. Title: A composition for preventing or treating osteoarthritis and uses thereof. Applicant: Industry-Academic Cooperation Foundation, Yonsei University. Application WO. The sequence listing filed with the application follows.

SEQUENCE LISTING (69 sequences)

SEQ ID NO: 1 - RNA, 5904 nt, Homo sapiens
  source 1..5904: mol_type = other RNA
cctttggtttgattggattcatcatgaggcagcatgggtttgcacttgtagaaatcaaaactgttaggtcaggtagtaaagccaatccttgaacttacatctttagttaaggcatcaaagaattgtaagttgctttgcaatgatgccatctccacatggtcagattcttccagtaaactgtgcagatattttacagaataagagctaagtttcagcatgtcaaggaatgatctgtactcaagtgttagtaaacaagggtttttttgtttgtttgtttgttttgagacagtctctgtcatccaggctggagtgcagtggcatgatcatagctcactgtatcctcagactactgggctcaagtgatcttcctgcctcagcctcctgcgtagctaagactacaagcgcatgccaccacccctggctaattttttattttttatggagaaggggtctcactatgttcccccaagctggtcttgaactcctggacttaagcaatcctcccacctcagcttcccaaagagttgggattaaaggcgtgagcccccatgtccggccaacaagacttcctcgtgactataatgtgagcataatattaatagctctgagagagagaagtgaaccagaagaccaacctcagtgtcaggaagtctgggcgtctgtcttctgcatggctgaagacatggggctttgggcaagtcatctgttctctttgaactttggcttcctcacttctgaaataggagggtcagagaagatgtttctttttgctgaaaagttttacagttctctgatctataccccttggtcacacacaaccaaaaagtagaaaacatgagtgcaatacttttccaccagtactcccagtttatacattatcttctcaaaccaataaggaacttctacaaggccctgttagtgatgtgttacaggtgccagcattagggaaactttcagactgttatatctattcgttccttcatccatgtatactattcattctgtatgcagagtaatttatatatgtacaattacatggcagtgaaagataatcagaaaaatgaagttttttttttttttttgagatagttttgagacagagtcttgctctgtttcccaggctggagtgcagtggtgtgatcttggctcactgcaacctccgcctcccgggttcaagggattctcgtgcctcatcctcccgagtagctgggactacagacatgcgccaccatacccagctaatttttgtatttttagtagagatggggttttgccatgttggccaggccattctcgaactcctggcctcaagcgatcctcctgccggcttcccaaagtaccgggattccaggcatgagccaccatgcccagtcagaaggtttttttttaaaaaacacactcctgaactaacaattacaaagagctagtgacaatttcccaaataattatgcataacaggagcccatatattgttctcaaatcataaaccataactgattttgaggaaaagacattctgtcccactgatattcttttcatgagtaagatctggatctgtctggaggcacagaattaatttttgcatgaggaatcccaaccctaccatcattccatggctgaggaattggttattactcctatgggaaattgggaatgttgttggtaccccagccttctcttaagacaaaatttaacaaatgcatacatgctaagatgcttatactcataaggctttgtgggtctcctttctaaggggaatttgaatactaacaagaacaaaggctaaataccaaaagggggctttctaatggtagaatttgggatatcaggtagccacatagagcagggctactttgggggctggagactgcagaaacccttcagtttatacgtgtgagtaaacctaatcacacttgatgtattgctagtgaagtcccagccccctgagcctttgcagaaacccaaagaatgctaaaaagggcaggttttagttcctgccaattatttcatttactacaaatgccccgagttccgaatttacttccctccccaccagaaatatgtcattttggaggcttgtgaaaattaagcattaagaaaatcccgcctccatcctaatacactgcatccacaagtcccaaacaaaatcacttccttggcctacacacataactacctgtttctgtttaggtctgtgactcagaaagtgcctggaagaagtcatgagagggagtcgatcccatcttacctgccataggaagaatagggcctgctcagtagagttcagtgtgtgtgttgaaggtggtggttcttagtccttccctgaattcactaattcgcattgcactcactcttcctgatcaatgagttattgctgagaaatcattgtagtaagtaatacaggtatccccagtaaagccatccctctcctccatacctccgctgtcccttgggttttggctccaggatccttgccccatgtcccaaagaatccctaccttgggcctccctcctcctcttttgtcaattgcacttgaccttttcaggaaaaagaaatcaattgataccttagtcctaatgtttgacccttttctatctcagaatagagaagtccctgtatttgttctttttttactcaagtttaatatagaccacctaggcacagaagctccgtgctatattctgttgcctgtaattgtccttccatctaattgggaaaaggttactctattgaaccatctgctgattcccttaccttttcactcttttgtcagtattcctttaccagtaaattcttggttatctaggtcctgaagtttcattcatgttttttttaaaagctttaatttttcttaggaaaactgtttctctcatcttaaagcagactatgatcttttctactttgttatacaatctgaacataatgaacactctaaagtcaggcatggattttatcataaaagcagatcgtattaagatttttttaaaaaagaaccaggattgaggaatctgtagctaataatttaataattcaccagcatgttttgggctcccacttcatgctggccactgggctaggcactgagggtgcagaagcaaacaaatcagcctcctggccctcagatttgcattccagtgagtccattcataaaacctaactcaaagccagcaacacccccaaaagggctgttggaagctttgtagctcatctgtacagctgtcttgattcctgtacgggatcttactttcttgggaaaatatgttctaaatcctgtttccttgggccattaaaaatccatgctgtccctaatcaatatatagttatgtgtgaccttcttagaattaaaaaaatgccgctggacagcctttgaagggaaaggcagagaaatctgttttgatggcttgaaaataagtgaaaaggtttttagggaaagctaacaagctttcaaagatttcagatctgccagcattcattcattaaggcatgggattaggccaaaagagcctcctaccaagggagagacaggaaccatgtaaggagatctgtgagaccgcagtggaagagtattgaaatagaagccagacctgtagacgtatttgttaatatgtgtgccaagccaaagtacaggaggaggcttggaggcatggagttgtggtggaagcaggttctgaaaagcagaactctgaagctggctcattctcacgaagtcatctggcccagcctcccgcctccaagcacatcctgcctgcagagggtctggctagctgccttttcagctctcgagggatagagattctacaacctccctctgtcatcagttccagagccactcccctttgcactagaagttcttgctttcaaagaatgagggtgtgagggagggaggggtcaagaaacagagtgacaggggaaacaggcagaacaagtcagggcaaaggaccccagcatgaagagttgtggaggtggaggtggggaagcagcctcacatctcacacttccttccttctcttaaatgtgagcagctgactccaagccttgtggaaactctagaaggtagaaccagccatctggggaagctggccttacagatgccccgtctggcatagtggaggttcctgtgctctgagaacgcagtgtgaatctagacatccactgcagcctgggaagagctgtgttttcttcaaaagtctttaactttcacagtcacccctctaaagaaatgttctctgattgaaggcatgcttctattcctactttattgtgtttcatgcattctgccagagtaattacttttcataccaattcttggatgcagagaaatctctggtagtctaaggggatttcgatccaagtaaagctactatctcctattccatccagacttttccgtctgcctccattctctcagtcacatacctagaagcaagccagaaagcctgtccaaccaaaatcactctccaaagcccaagcactttattgttctccctgtctgttatcgagccaaggtgtatttggcctcattttatgccattagttgtctggctttcatggctctgcaccacattacagtcagagcaggaaggccagcagtggagatagaattatggcagaaacccagagtagaggcctctgctggtgagggagcctgcagcactctccacgctggtgggtcctagcatgcccaacagacccccatcccttcccatcagccttgggccttgagtctcattccaactcatcccctcccctttcccttctttccagtcccaggtgacacttgatgcctctgactcctttgaagagggcatcaagaagtgaaagaacaaagtccttttctgttcgggatctgggcccatcctgggagaggtttttggcagaaatggctgcagtggaaccctctgactgccagggtgaaatagtgctccagcaggctgcggtagactcactgccagagtgggtcaggactggcccagaggacagggtcgtctcttgagagtcctcccagctccagggcctgattttaaagcagtaacacgaggatataggttatatacaggctcctggaaggcaggtgccgcagctcctgtgacaccccatatgcctgagcaagcttctccagcacaagagatgatgcaagtatgaatgggtacggggggagcttaaaacctgccaacactgagacttgatgccaggggccgtgcacccgctctgccacctgctaggtctgtgcaatggtcagagcagaggtgtgtgatgagttcagctcccaagcacatccacacttaggaagtgttctgtgtgtttttaaataatccttaccatgtaaagattgtattacatttgtatacaaaatttttttgcattttacttttgtaatatttggggttttatagatttttattttatggccaagtatacttttgtaaggaaatgttgaagtcttgagtatttttattcttttaaaaaactatagttagtgtcaactgtgagcactgataaatattattcatgtgtggttttccttctttttaatccagactttttaagaaactgttttggcatagagctttacttaaaatgctgcttcattttacacattgtgaatactgaagattctaaaaaataaagatgcatttaaaatctctgtgctgttccattgtagaaatggtaatgtgcattgctttgccaaagtggtaattaaatgtttaatggtttagaactcctagttcacaacagggcttctcgtcatcacttgcagcgtgtgagcttccaaataagccgccatttctttggaaaacgcacgcacttaggcatggcgatctcctgttccgttaggaaatacggttatgttgacattatggttactgtgcttgtggttttgcaataaacatgtattgaaagca

SEQ ID NO: 2 - RNA, 2344 nt, Homo sapiens
  source 1..2344: mol_type = other RNA
gcttctgacccgggccgagccgggaactcagcgccagctctgttcctggcggggctgaggcttccctcacattccaggccacctggcaaacgtcctgaggctgccactccttctgggctcaaggctcacgggctgaggtctgtccccgcgtggagctcaaggctcacgggctgagtgcctgagaagaaaacagaactgccagcagactatgggacaaacgactaaatgccctccagacgttccagagtcctctgcctctcaggcttcagttcttcctgaaggaatctggagctggaaagcaggaagcaatttgctgtggaattttttccatcacagactccaagttcctcagcctttggactcttgaacttacaccagtgttttggcaggagcgctcgggcctttggccacagactgaaggctgcattgtcagcttccctacttttgaggttttgggactcagactgatccaccactggcttccttgctcttcaacttgaagacggcctatcgtgagactttacctcgtgattatccttgcctggattctccacctcctcaaccccaggaagcaacaagctatcaaagacagaatttgcacaacaggacaaaggaaggctataagcttcttgaaggcagagattatatctcattcaatcttctatctcaagtatctactgcaaaaccaagcaaacggcgatctgagcacctgatggcagaactggaagaggtgaaagaaaaccccagggacactctggacatgttctgtattatttggatccagactggtctgaatttatcaaaagagattaacatgatataaaccaagagggaaatgaagaaacgaagcatgttcattttggattgaagaaaagtttgtcattataatgtatcttcagatttggttgccgtgcagggcaatttactgttcttttgatctttttctctgtttaaaaagacatggactaggcgaggaatggagcaggtgaagcaccgctgacattattagtgtgcgtgtgaacctctgatatgctaataggcaaagtgggtggaatggaattgctcttaaataagtaaaaaacttaacattcaattacctttaaaaatgggcataatttggagggtttcatttaacacactgcaggtaaaatctaattttgtttttctaaactttcctttgctaatgcaaggcaggagagttttgtgtgtgtttaaatagaccaaagtctcactggggagagtcagaggtctgggattctcatattttggagatagtaatttgattttcctaggatccttttttttttttttttttagcagaaaaatgtggtaacagtgtcatccagtcacagccatggagacgacccagtagggattcatagaattttgcaaatgctcctctgtcccgtgagatgaaattcctttcccatccaaagtacccacccaaagagaaaactatcctaggacttttgcttcttccagaaattacttcagacatctccccctttcagactctctctctttcccctgctgtttcatttcctctggttgtagtaatgtagaaaccctttgtgtcgtgcaggggctaagagcgtgctctctgaagccacgcagcctcccagacagtctagacactgctgttgatgaactgtaccatcttgattatttcactgaacccctttgaggttttcctcacatagaaaatggggatagtaatagttcctactgcctagtgttgttttgaagattaaatgaaactgtgcatgtaaagtggtaagcaccaaatggtgttagcagttgttattgttgctattattattactattacttttaacttgtaggtgtttgagccaagcccagggcctcctgcatgtgccagcttcagtagctgcaccagcagtccccattgggcactgtggcagtggtggtgatggaggaggaggtggtggtaaagaggggaacaagtggattaagcagagggaggtgaggcaggaggaaggcatgatgggagggtaatatggttaggctttgtatccctacccaaatctcatcttgaattgtaattcccaggtggttagggagagactggtgggaagtgattggattatgggggcagtttcctacacgctgttctcatctcgtggtagtgagtgagttctcgctagatctgatgattttataaggggctcttcccgcttcaatcctcatactctctctcctgccgccatgtgagggaaggtcttagcttgcttctcctttgccttctgccatgattgtaaatttcctgaggcctccgcagccatgtggaactgtgagtcaattaaacctctttcctttataaatt

SEQ ID NO: 3 - RNA, 1506 nt, Homo sapiens
  source 1..1506: mol_type = other RNA
ccgagtgcagagccagggcccagcacgaaggccttgggctccagtccgtgtgccccacatccctacatgagtgagggtggagggatggtgcctctgccacggccacggtgccgccgtccacgtcagctcactctcagcacaggtgctgtgtgacggcctcgggccacaccgcttgttctgaggcccctagcaggtcgggcttgtgctggctgcacattggctggtgagcttggcgggtctgtgggcacggagagaccagaacgtgcgtaacaggcccgatgagggtgccaggctgtggcgacccccgagcttcagaggagaggggcaccagccgggggccctgcacaggcagcctcagagagaggaaagctcacgatctgggagaactccaggcctggcccagtgaagacgtccttatcttcagcagacattgcccagtgcaaggggagggatttttagggcggcaagctcaggtggacaggcagttttattctgtttcccatgtcaagtccagccccagactgactttctgaggtcacagacggagcctcaccccatccaaggcggtgtcctggactcccactgtgctccccagagggcagggtacctggggcccagcccgggcggcaggagggactcagcccctcgcccaggcaggaagggtcccaagcagaggcccctccctcaggcactccccagcccacacctgcagcactgggaccaagactaataaaacaccagcctcacggaagacagctttatcttgttgatcggaagtctgccagcccaatttatgatggaacataagatctctaaatctgaatttacgctctgtagcgtaacgagaggtcaataagattaaacgggggctcaggagaggaccagcgtcaggctcactgcgaggtgctgcacagaaaacccacagccagagcccctgggcccagcccaggcaagaccagaaaaggagggggcaggtgggagaccagcctggggctcccgggaagcccacgggatggaggcgggagagccaggaggcctggggcaaccctgggacggttcctggatcgaggagagcaggggggtgatgagggttccctcagggctggggagccttctcctggtctcagacccaccccccttcagctcccaagccctgggtgcccctggctctgaggacagttgggaatcttccctgaggcaggttcaaggacagagctctgaccctggcccagggctgctttgggtgcctatgaactcggcttctggctcagagcagttccctgcaccccttcctgagccctctgtcctctggaacccgtgggcagggtgagggacgggtgttccttctgggtgggggcctgggcgcccagccagcacgacgctggcttgctgagcttagggcagaccccgacttcagaatttatacaaataaatgcaatgaaaagtgctggcaacctgatctgattacagagtcattcattctctggtcgttaataatttgtgcaa

SEQ ID NO: 4 - RNA, 2719 nt, Homo sapiens
  source 1..2719: mol_type = other RNA
gcggggggatcgggtagctctggcggaggctgcgcccccggcgtgctcgggcagagaagaacggaggcccgctgaggatgggaactcaggctccgggtctgggacacaataatccggccgaaggcgagcggccacactggactaggaaacgaggcgccgggctgtaaggtgggcccgcgccttttctcctgcctggcgctgattcccgcatttttcgctcgcgccctgcgctgcgcgctgcctgtgcgcctccctgggcgcgcgggcgggagagtcgggcgagcgccaagacggctgggcccgactcccactggcgccccggctccacctggcgctggggctccggtccgcagtggctccggcaggagggagagaacgaggagggaggcttggaaacgccgggagtagcggtgaggccgacgccggggaagcgaatcgatactgcgttactggacgcccgtgggcctcatgaggatggtcgattccctcattcgttattcacgatttattagggatggcggccgcgtctgtccctccagagagctcgattatccatccggccagcagcgccattaagcgcactgacggtgggaggctcgagttagaaattaggataggaatcttcgcccagttttggagcgcctgcctcctcttccctcgttgctcgcagccaaggcagccgcgaagctgggggcctcgggtgaatgctttcgccctctggccggcgaccaggagacctgcgcacactggccgccgagtgaccccagctcgagcctgcagccacaccagcgggacgggggcggggaggaagaggaagggcggagagacttccttccagagggagtggtccgagaaccggcgggagaagggccaagggaagatccggtcacctgctccggagcctgcaggcggagaggcgagtagttcaccggccccggaggaaaggggaccctcccactgttcccaggcaaatgtgtcgccggcatcctgcactctgccggggaagacgcgcatccactcgctctgcagggaggggaacgcgggaaggactcccagtcagccgcccctctctggctacaagaccccgaacaagagaaacctgtaacaggggctctgcggagatctggatcccacccaccaaccacatgggcacctggggggctgcccctcggggcattatcagccagtgggaagggggttgacgttcctctgcggcccatgaatcctggagggctgcccgaggggccaccggggtccatccacttattcttcggttgttaagcgccagacaggagagaaccgctagagaggagtgtgctaagaccctattacccactaaaactccattttcatcttttgcgtcctggatgactagtctccacattcctggcctttctggtttctcaggagaaccttctgacccaactcttcccacatcgaaagagtttcctagtcttttgttctactactagccgacatagaaagcacctgtcatgtgccagtgtcaaatactgcgctaggaactgggaactcaaggcacaggagcctggcttttgcgcagggcgctcacaggccggtgggtgcaaaccctgaaggacacacagcctgtccctttagcgcccatcgcttctggtgtgagctcccgctaagggtgggtgagtactggggtgggcttccagaagaggcctcctttgagccgaatctgcagagaccaagtgtctatgagaactgctcaagagtgctttgcacattctcctccacaaaggtcgaggctcccactgcgcccaggaatgcgcctcgtcagacattaggcgccccttgattttgtgtttgcatctcacgcggtcctctagctgacaagtgcatcagaagagtcacagtggctgtcacaagccagagactcgcagaggacaggaacgcgggaaatctaggcaattacctccagcatataccaagagctattgcgaggatcagatccctttaaaaatggtgacgagacaggagagggcggctcctctagagctttccggaacgtctttacctctgtgtcctttataccttttatctcccccaaacaaggtccttagtcagtttctccttctatttccccatcttcctcccccacctccctgtgtagttctagggggaaaaaatgtgttgttttcctttttttctgatgcttctaatattaaatgcgtctattttcccactctccattgtcttgaggtcttcccctacccaccctgcctagttctgtcacgtcccttctttccctgtatcacaacaatgttctccctttctcacctttgtttctcttcatacttgtttctctctctgtgtctctctcattctcttcccttccaaatgtagtatttggagactgtaatatcgattgaggcagacaatagaaaactgtcgaacctccactgtaaattcattcttaatcctatgaaaaaatgcatcctgaaacgtgttgcatgcacagtgagacaaaaacctgtgtctttaggtttcctgcgatctagcttggaggcgggttgggggggtgtggagggaagtgctggagaaattatcccattattgactgagcagcaaagaattttcaagaacagtgattctcctagaaaaagtattgctgctgccatttcaatgcaaaatttggcttttgagtaaaaggcttaggtttttatcttccggggagaaaaaaaaaacccaaaag

SEQ ID NO: 5 - RNA, 543 nt, Homo sapiens
  source 1..543: mol_type = other RNA
caggtgctggccctttgcctgtgatgtggtgtccctctttctctctcttgtccccccagctcagggccctacccccagcactcacctgaggcccgacctccaagcaggcctgggagggaagggctgtataccgttgccatggataccagcacccagaaggggtggggctgtttgttaccaggagcctccagggagaccccagaccaggcccctagagacagggtcttgctccgctgtccaggctggaatgcttcggtgtgatgacagcgcacgttaacctcgaattcctgggctcaggtgatcctcccacttccgcctcctgacttgctgaaactacaggcacccgcctccaccgccaggcccagcccacagctcctttgacctcagtgacaggcactcacctacctgacccccaaactgaagcctcacttttcccagccgtgtccacaccctctgggctaccccattaccatgacaagtattccctctgctccaggagaaaagccaggtcccagacctgacccattaaaacccaatcattcc

SEQ ID NO: 6 - RNA, 2624 nt, Homo sapiens
  source 1..2624: mol_type = other RNA
caagtcgcagccatacattatctggagggtgttagaccctggccccgcccccgcggtcagccccgcccaccgagccccgcccccgccccgaccaacccgcggggattttggcctaaacggaaaatgaaacctggtaaaggcgcctgggcctctcccgggtcgaggatctggcgggtcccgcagcctcggggtggatcttggagccggagactcgcgggggggacccgggacgtccgtgggggatgaggaggggtcgtgaccttcgccccaggccggggtcattcaccggcctagctctggtggtagtagcggcgcggcatgggcaggttcactcttgtcagtctgtgcgcgggcctgatgttccgtgtgctccggtcccaatactccggtccctcctgctccaaccacggcgactgcggctacatcctcggagtcgccgcgtcgctgtcgaaccgcacgaactgcgtgtcgtccacgtagcccactgcgatgtaccggggctccccgcgacccggccgggacacggcggtgctgaaataccttatggagtgggtacctgggggcgaggaggggctgagacccgtccgaccctcctccttgcgctgctccccgggtcctgcgccccagtgcgcgggcccctacctcctccccgcagaggccatttccctccggatcccgcactcacccgcccaggtctcggtcagggccagggcccccaagagcagcaggaggagggttcgggacgccatgaccccatcctcggcgtctggggagaatctgagtcccaatgggttcgcggggacttctggaacagggaccccagcgacgccgattggcttcgctagaaacccgacaccaaatgggggtgagaactgagtccacatcctgagtgtccaggaagaaggaccctacataagttgggagagggagaagagaaactgcggagatggggaatccccaaccctgggcctccccaatcaatacatcgccttcggggcctgaaaccctgagagccacgcctggggccataggacttcgccctgaccccgctcctcctgtgccaagcgctctgtctcaatgtctccctgagtcttggcccaagagctgtctgagaaaccagggagaaaccctcgtcatgggccccgtccctcttcatttttcatcccggaatccccgtcccagaactggactccctgcctcccactccttacctatttccctgaactcttctagaaaaaaactcaccccagggagcttggtgacagagagggagctcgccgccagagagggagctcgccgccagagagggagctcgatgccagagagggagctcgccctgggaatggaggcgtagagacaggtttttgttttttttttctttaaatccggaaaagttgtgcctgagtacatgagacagcatagagacaagttttctctttgtttattaactacagtgggtagcagaatcttggcaacccctaaatgatcaggtatctaatcggtaaaaaaatgtaactttggccccttgatacataaatgtgtctgaaagcattacaacaggactcacaaagctactaagtttgactttcgcagacaatgtatctgtgactcccgcttgttttttacatttaccttcattccacagccctgagttactgggtgagtccaagacatctcctcaatataaagtagcacactgcgttactatatgttgcaaccgggagccagtacagactttattcacctcacagttgcaagtgttcaatgcagtcacaatgcccctcagcagtgctcatgtgctgcctgtttttaggaagtattcacgtctaagtggtgtgtatatcttataggaacacttagtatttttaaaacctgattaattaaaaaaaattagtttctaggcagtcccaaatatagtattaaaggccaactgcaaagaaggaacactaagtgttttttaaaccttattaacataaaaaacattagtttttaggcagtcctacattaggtattaaaggccaactgcaaagaacactgagcgaggctctgtagatggatgtaataaaaatctataaaacaatgtgtttaaacctaagaattctactgctttccaattccttccctctgctccttttcctaacctcctgcttctccagcccttccctctgtccctttcatccctcaggccctcctctccccttagtccccaccaccctgtcacttctaaattgtggctctagcattgtcccattacctgctacgtgactgttctctccacagtggtcctgctcctgtgagtcagagtgtgtcatttcctcacctaaaacactccagtggctccacctcggtcttgtgaagcttctagaatgtcaggcacgtgagcatatgagggcatacctggttcatcttaggcactaaatttttgttgactgaatgaatgaaatatgaatgtattaaattgcatcacagaaagttataaaatgtaaaacactgaaaaattaagaaatattttattttatgtaactagtgtgcatatcaattcattccgagtctgttgagcctgtgtatgaattttataagattgcataacaaattatcacaaacattgactttaaacaacaccc

SEQ ID NO: 7 - RNA, 471 nt, Homo sapiens
  source 1..471: mol_type = other RNA
gtctcgcggtgccccccagtgccggaggggaaggagcgggcgtgaaggacgcgagctggaggacagtctcgattcgggcctgagccgtggaagccgttggccttcgcacaggaaagaggagcccgagatcagtctctctgcgcctccctgcttccccccttgaatggagctgcgttcaggagctgcctacagtgcccagcgcatggcagccatgctgaggaggggtacagggccaagagacacctgggtcagaagcttccctgagggcctcccaacaggaagactctgggccctgccgcccacccgccacagctccgttttcagccacagcatccctgacctctccttggagaatgtgggggccactggacacgccaggccctgatgccggcacaggcagcctcctcttgttcctggaccaaactgagagtcgggctgctatttctcgtggcccagtaacgagatgcagat

SEQ ID NO: 8 - DNA, 19 bp, synthetic construct
  source 1..19: mol_type = other DNA
ccgagcttcagaggagagg

SEQ ID NO: 9 - DNA, 20 bp, synthetic construct
  source 1..20: mol_type = other DNA
ctcccagatcgtgagctttc

SEQ ID NO: 10 - DNA, 19 bp, synthetic construct
  source 1..19: mol_type = other DNA
ggtgccgaagacctgagac

SEQ ID NO: 11 - DNA, 23 bp, synthetic construct
  source 1..23: mol_type = other DNA
ggccacttcttcattcttgttgg

SEQ ID NO: 12 - DNA, 20 bp, synthetic construct
  source 1..20: mol_type = other DNA
gtcattcaccggcctagctc

SEQ ID NO: 13 - DNA, 20 bp, synthetic construct
  source 1..20: mol_type = other DNA
gagtattgggaccggagcac

SEQ ID NO: 14 - DNA, 20 bp, synthetic construct
  source 1..20: mol_type = other DNA
gaagcaagccagaaagcctg

SEQ ID NO: 15 - DNA, 20 bp, synthetic construct
  source 1..20: mol_type = other DNA
gtggtgcagagccatgaaag

SEQ ID NO: 16 - DNA, 20 bp, synthetic construct
  source 1..20: mol_type = other DNA
gatcagtctctctgcgcctc

SEQ ID NO: 17 - DNA, 20 bp, synthetic construct
  source 1..20: mol_type = other DNA
gtgtctcttggccctgtacc

SEQ ID NO: 18 - DNA, 20 bp, synthetic construct
  source 1..20: mol_type = other DNA
caggcactcacctacctgac

SEQ ID NO: 19 - DNA, 22 bp, synthetic construct
  source 1..22: mol_type = other DNA
cctggagcagagggaatacttg

SEQ ID NO: 20 - DNA, 20 bp, synthetic construct
  source 1..20: mol_type = other DNA
actgggaactcaaggcacag

SEQ ID NO: 21 - DNA, 20 bp, synthetic construct
  source 1..20: mol_type = other DNA
agattcggctcaaaggaggc

SEQ ID NO: 22 - DNA, 21 bp, synthetic construct
  source 1..21: mol_type = other DNA
gcacaacaggacaaaggaagg

SEQ ID NO: 23 - DNA, 19 bp, synthetic construct
  source 1..19: mol_type = other DNA
cagatcgccgtttgcttgg

SEQ ID NO: 24 - DNA, 20 bp, synthetic construct
  source 1..20: mol_type = other DNA
aagaaatggtgctacccagc

SEQ ID NO: 25 - DNA, 20 bp, synthetic construct
  source 1..20: mol_type = other DNA
gtgcagtggttgtaaagtgc

SEQ ID NO: 26 - DNA, 19 bp, synthetic construct
  source 1..19: mol_type = other DNA
ctcctcgatgccgtacttg

SEQ ID NO: 27 - DNA, 20 bp, synthetic construct
  source 1..20: mol_type = other DNA
ccacgttcctatgtgaggtg

SEQ ID NO: 28 - DNA, 20 bp, synthetic construct
  source 1..20: mol_type = other DNA
cctcctaccaattacacgcc

SEQ ID NO: 29 - DNA, 20 bp, synthetic construct
  source 1..20: mol_type = other DNA
gtacacacaggtcgctatgg

SEQ ID NO: 30 - DNA, 20 bp, synthetic construct
  source 1..20: mol_type = other DNA
ttaaacgagccctggatctg

SEQ ID NO: 31 - DNA, 20 bp, synthetic construct
  source 1..20: mol_type = other DNA
cccgaaacagacttctgaac

SEQ ID NO: 32 - DNA, 20 bp, synthetic construct
  source 1..20: mol_type = other DNA
atcgctcgccaactacagac

SEQ ID NO: 33 - DNA, 20 bp, synthetic construct
  source 1..20: mol_type = other DNA
tggcttctcgctccactttc

SEQ ID NO: 34 - DNA, 20 bp, synthetic construct
  source 1..20: mol_type = other DNA
gggtagcatagtgcccaagg

SEQ ID NO: 35 - DNA, 20 bp, synthetic construct
  source 1..20: mol_type = other DNA
tttattggagagggccgctg

SEQ ID NO: 36 - DNA, 20 bp, synthetic construct
  source 1..20: mol_type = other DNA
ttgctgatgacgcagaggtc

SEQ ID NO: 37 - DNA, 20 bp, synthetic construct
  source 1..20: mol_type = other DNA
ggacattattgccgccgttc

SEQ ID NO: 38 - DNA, 20 bp, synthetic construct
  source 1..20: mol_type = other DNA
gagagcgagcttcggaaagg

SEQ ID NO: 39 - DNA, 19 bp, synthetic construct
  source 1..19: mol_type = other DNA
ttcctttgaacggcgtcgg

SEQ ID NO: 40 - DNA, 19 bp, synthetic construct
  source 1..19: mol_type = other DNA
ctcccaacctcacctgtgc

SEQ ID NO: 41 - DNA, 20 bp, synthetic construct
  source 1..20: mol_type = other DNA
tagcagggctttggatgtgc

SEQ ID NO: 42 - DNA, 21 bp, synthetic construct
  source 1..21: mol_type = other DNA
agcaccctaacgacaacagtc

SEQ ID NO: 43 - DNA, 21 bp, synthetic construct
  source 1..21: mol_type = other DNA
agaacccagctccattcatcc

SEQ ID NO: 44 - DNA, 20 bp, synthetic construct
  source 1..20: mol_type = other DNA
ttacaggtgtctgtgcggtg

SEQ ID NO: 45 - DNA, 21 bp, synthetic construct
  source 1..21: mol_type = other DNA
tccagtcaatccttggcatcc

SEQ ID NO: 46 - DNA, 20 bp, synthetic construct
  source 1..20: mol_type = other DNA
atctcagggtttcccacgtc

SEQ ID NO: 47 - DNA, 20 bp, synthetic construct
  source 1..20: mol_type = other DNA
actgtccaggctttcaggag

SEQ ID NO: 48 - DNA, 20 bp, synthetic construct
  source 1..20: mol_type = other DNA
acagccgggaagaaaattgt

SEQ ID NO: 49 - DNA, 20 bp, synthetic construct
  source 1..20: mol_type = other DNA
ccagaagttcatggcagcag

SEQ ID NO: 50 - DNA, 21 bp, synthetic construct
  source 1..21: mol_type = other DNA
gtcctctcccaagtccacaca

SEQ ID NO: 51 - DNA, 21 bp, synthetic construct
  source 1..21: mol_type = other DNA
gggcacgaaggctcatcattc

SEQ ID NO: 52 - RNA, 19 nt, synthetic construct
  source 1..19: mol_type = other RNA
cctacgccaccaatttcgt

SEQ ID NO: 53 - RNA, 19 nt, synthetic construct
  source 1..19: mol_type = other RNA
acgaaattggtggcgtagg

SEQ ID NO: 54 - RNA, 19 nt, synthetic construct
  source 1..19: mol_type = other RNA
caggattgaggaatctgta

SEQ ID NO: 55 - RNA, 19 nt, synthetic construct
  source 1..19: mol_type = other RNA
tacagattcctcaatcctg

SEQ ID NO: 56 - RNA, 19 nt, synthetic construct
  source 1..19: mol_type = other RNA
cagaactgccagcagacta

SEQ ID NO: 57 - RNA, 19 nt, synthetic construct
  source 1..19: mol_type = other RNA
tagtctgctggcagttctg

SEQ ID NO: 58 - RNA, 19 nt, synthetic construct
  source 1..19: mol_type = other RNA
gattacagagtcattcatt

SEQ ID NO: 59 - RNA, 19 nt, synthetic construct
  source 1..19: mol_type = other RNA
aatgaatgactctgtaatc

SEQ ID NO: 60 - RNA, 18 nt, synthetic construct
  source 1..18: mol_type = other RNA
caattacctccagcatat

SEQ ID NO: 61 - RNA, 19 nt, synthetic construct
  source 1..19: mol_type = other RNA
tatatgctggaggtaattg

SEQ ID NO: 62 - RNA, 19 nt, synthetic construct
  source 1..19: mol_type = other RNA
ctgacttgctgaaactaca

SEQ ID NO: 63 - RNA, 19 nt, synthetic construct
  source 1..19: mol_type = other RNA
tgtagtttcagcaagtcag

SEQ ID NO: 64 - RNA, 19 nt, synthetic construct
  source 1..19: mol_type = other RNA
ctgcaaagaaggaacacta

SEQ ID NO: 65 - RNA, 19 nt, synthetic construct
  source 1..19: mol_type = other RNA
tagtgttccttctttgcag

SEQ ID NO: 66 - RNA, 19 nt, synthetic construct
  source 1..19: mol_type = other RNA
gcagcctcctcttgttcct

SEQ ID NO: 67 - RNA, 19 nt, synthetic construct
  source 1..19: mol_type = other RNA
aggaacaagaggaggctgc

SEQ ID NO: 68 - RNA, 19 nt, synthetic construct
  source 1..19: mol_type = other RNA
gactctcttcatatggact

SEQ ID NO: 69 - RNA, 19 nt, synthetic construct
  source 1..19: mol_type = other RNA
agtccatatgaagagagtc